European Patent Specification EP 3 733 692 B1, published August 21, 2024. Title: ANTAGONIST PEPTIDE OF THE INTERLEUKIN-15 ACTIVITY. Applicant: CENTER OF GENETIC ENGINEERING AND BIOTECHNOLOGY. Application CU 2017-0177. The sequence listing filed with the application follows.

SEQUENCE LISTING (13 sequences)

SEQ ID NO: 1 - protein, 10 aa, Homo sapiens
KVTAMKCFLL

SEQ ID NO: 2 - protein, 10 aa, Artificial Sequence
  Description of the Artificial Sequence: Peptide 2-Lys 1 is a D-amino acid
KVTAMKCFLL

SEQ ID NO: 3 - protein, 10 aa, Artificial Sequence
  Description of the Artificial Sequence: Peptide 3-Val is a D-amino acid
KVTAMKCFLL

SEQ ID NO: 4 - protein, 10 aa, Artificial Sequence
  Description of the Artificial Sequence: Peptide 4-Thr is a D-amino acid
KVTAMKCFLL

SEQ ID NO: 5 - protein, 10 aa, Artificial Sequence
  Description of the Artificial Sequence: Peptide 5-Ala is a D-amino acid
KVTAMKCFLL

SEQ ID NO: 6 - protein, 10 aa, Artificial Sequence
  Description of the Artificial Sequence: Peptide 6-Met is a D-amino acid
KVTAMKCFLL

SEQ ID NO: 7 - protein, 10 aa, Artificial Sequence
  Description of the Artificial Sequence: Peptide 7-Lys 6 is a D-amino acid
KVTAMKCFLL

SEQ ID NO: 8 - protein, 10 aa, Artificial Sequence
  Description of the Artificial Sequence: Peptide 8-Cys is a D-amino acid
KVTAMKCFLL

SEQ ID NO: 9 - protein, 10 aa, Artificial Sequence
  Description of the Artificial Sequence: Peptide 9-Phe is a D-amino acid
KVTAMKCFLL

SEQ ID NO: 10 - protein, 10 aa, Artificial Sequence
  Description of the Artificial Sequence: Peptide 10-Leu 9 is a D-amino acid
KVTAMKCFLL

SEQ ID NO: 11 - protein, 10 aa, Artificial Sequence
  Description of the Artificial Sequence: Peptide 11-Leu 10 is a D-amino acid
KVTAMKCFLL

SEQ ID NO: 12 - protein, 10 aa, Artificial Sequence
  Description of the Artificial Sequence: Peptide 13-Lys 1 and Ala are D-amino acids
KVTAMKCFLL

SEQ ID NO: 13 - protein, 10 aa, Artificial Sequence
  Description of the Artificial Sequence: Peptide 15-Ala and Cys are D-amino acids
KVTAMKCFLL